European Patent Application EP 4 119 168 A1, published January 18, 2023. Title: METHODS FOR THE TREATMENT OF DANON DISEASE AND OTHER DISORDERS OF AUTOPHAGY. Applicant: The Regents of the University of California. The sequence listing filed with the application follows.

SEQUENCE LISTING (12 sequences)

SEQ ID NO: 1 - DNA, 1233 bp, Homo sapiens
atggtgtgcttccgcctcttcccggttccgggctcagggctcgttctggtctgcctagtcctgggagctgtgcggtcttatgcattggaacttaatttgacagattcagaaaatgccacttgcctttatgcaaaatggcagatgaatttcacagttcgctatgaaactacaaataaaacttataaaactgtaaccatttcagaccatggcactgtgacatataatggaagcatttgtggggatgatcagaatggtcccaaaatagcagtgcagttcggacctggcttttcctggattgcgaattttaccaaggcagcatctacttattcaattgacagcgtctcattttcctacaacactggtgataacacaacatttcctgatgctgaagataaaggaattcttactgttgatgaacttttggccatcagaattccattgaatgacctttttagatgcaatagtttatcaactttggaaaagaatgatgttgtccaacactactgggatgttcttgtacaagcttttgtccaaaatggcacagtgagcacaaatgagttcctgtgtgataaagacaaaacttcaacagtggcacccaccatacacaccactgtgccatctcctactacaacacctactccaaaggaaaaaccagaagctggaacctattcagttaataatggcaatgatacttgtctgctggctaccatggggctgcagctgaacatcactcaggataaggttgcttcagttattaacatcaaccccaatacaactcactccacaggcagctgccgttctcacactgctctacttagactcaatagcagcaccattaagtatctagactttgtctttgctgtgaaaaatgaaaaccgattttatctgaaggaagtgaacatcagcatgtatttggttaatggctccgttttcagcattgcaaataacaatctcagctactgggatgcccccctgggaagttcttatatgtgcaacaaagagcagactgtttcagtgtctggagcatttcagataaatacctttgatctaagggttcagcctttcaatgtgacacaaggaaagtattctacagctcaagactgcagtgcagatgacgacaacttcctagtgcccatagcggtgggagctgccttggcaggagtacttattctagtgttgctggcttattttattggtctcaagcaccatcatgctggatatgagcaattttag

SEQ ID NO: 2 - DNA, 1233 bp, Homo sapiens
atggtgtgcttccgcctcttcccggttccgggctcagggctcgttctggtctgcctagtcctgggagctgtgcggtcttatgcattggaacttaatttgacagattcagaaaatgccacttgcctttatgcaaaatggcagatgaatttcacagttcgctatgaaactacaaataaaacttataaaactgtaaccatttcagaccatggcactgtgacatataatggaagcatttgtggggatgatcagaatggtcccaaaatagcagtgcagttcggacctggcttttcctggattgcgaattttaccaaggcagcatctacttattcaattgacagcgtctcattttcctacaacactggtgataacacaacatttcctgatgctgaagataaaggaattcttactgttgatgaacttttggccatcagaattccattgaatgacctttttagatgcaatagtttatcaactttggaaaagaatgatgttgtccaacactactgggatgttcttgtacaagcttttgtccaaaatggcacagtgagcacaaatgagttcctgtgtgataaagacaaaacttcaacagtggcacccaccatacacaccactgtgccatctcctactacaacacctactccaaaggaaaaaccagaagctggaacctattcagttaataatggcaatgatacttgtctgctggctaccatggggctgcagctgaacatcactcaggataaggttgcttcagttattaacatcaaccccaatacaactcactccacaggcagctgccgttctcacactgctctacttagactcaatagcagcaccattaagtatctagactttgtctttgctgtgaaaaatgaaaaccgattttatctgaaggaagtgaacatcagcatgtatttggttaatggctccgttttcagcattgcaaataacaatctcagctactgggatgcccccctgggaagttcttatatgtgcaacaaagagcagactgtttcagtgtctggagcatttcagataaatacctttgatctaagggttcagcctttcaatgtgacacaaggaaagtattctacagcccaagagtgttcgctggatgatgacaccattctaatcccaattatagttggtgctggtctttcaggcttgattatcgttatagtgattgcttacgtaattggcagaagaaaaagttatgctggatatcagactctgtaa

SEQ ID NO: 3 - DNA, 1236 bp, Homo sapiens
atggtgtgcttccgcctcttcccggttccgggctcagggctcgttctggtctgcctagtcctgggagctgtgcggtcttatgcattggaacttaatttgacagattcagaaaatgccacttgcctttatgcaaaatggcagatgaatttcacagttcgctatgaaactacaaataaaacttataaaactgtaaccatttcagaccatggcactgtgacatataatggaagcatttgtggggatgatcagaatggtctcaaaatagcagtgcagttcggacctggcttttcctggattgcgaattttaccaaggcagcatctacttattcaattgacagcgtctcattttcctacaacactggtgataacacaacatttcctgatgctgaagataaaggaattcttactgttgatgaacttttggccatcagaattccattgaatgacctttttagatgcaatagtttatcaactttggaaaagaatgatgttgtccaacactactgggatgttcttgtacaagcttttgtccaaaatggcacagtgagcacaaatgagttcctgtgtgataaagacaaaacttcaacagtggcacccaccatacacaccactgtgccatctcctactacaacacctactccaaaggaaaaaccagaagctggaacctattcagttaataatggcaatgatacttgtctgctggctaccatggggctgcagctgaacatcactcaggataaggttgcttcagttattaacatcaaccccaatacaactcactccacaggcagctgccgttctcacactgctctacttagactcaatagcagcaccattaagtatctagactttgtctttgctgtgaaaaatgaaaaccgattttatctgaaggaagtgaacatcagcatgtatttggttaatggctccgttttcagcattgcaaataacaatctcagctactgggatgcccccctgggaagttcttatatgtgcaacaaagagcagactgtttcagtgtctggagcatttcagataaatacctttgatctaagggttcagcctttcaatgtgacacaaggaaagtattctacagctgaagaatgttctgctgactctgacctcaactttcttattcctgttgcagtgggtgtggccttgggcttccttataattgttgtctttatctcttatatgattggaagaaggaaaagtcgtactggttatcagtctgtgtaa

SEQ ID NO: 4 - protein, 90 aa, Homo sapiens
WDAPLGSSYMCNKEQTVSVSGAFQINTFDLRVQPFNVTQGKYSTAQDCSADDDNFLVPIAVGAALAGVLILVLLAYFIGLKHHHAGYEQF

SEQ ID NO: 5 - protein, 90 aa, Mus musculus
WDAPLGSSYMCNKEQVLSVSRAFQINTFNLKVQPFNVTKGQYSTAQDCSADEDNFLVPIAVGAALGGVLILVLLAYFIGLKRHHTGYEQF

SEQ ID NO: 6 - protein, 90 aa, Homo sapiens
WDAPLGSSYMCNKEQTVSVSGAFQINTFDLRVQPFNVTQGKYSTAQECSLDDDTILIPIIVGAGLSGLIIVIVIAYVIGRRKSYAGYQTL

SEQ ID NO: 7 - protein, 90 aa, Mus musculus
WDAPLGSSYMCNKEQVLSVSRAFQINTFNLKVQPFNVTKGQYSTAQECSLDDDTILIPIIVGAGLSGLIIVIVIAYLIGRRKTYAGYQTL

SEQ ID NO: 8 - protein, 91 aa, Homo sapiens
WDAPLGSSYMCNKEQTVSVSGAFQINTFDLRVQPFNVTQGKYSTAEECSADSDLNFLIPVAVGVALGFLIIVVFISYMIGRRKSRTGYQSV

SEQ ID NO: 9 - protein, 91 aa, Mus musculus
WDAPLGSSYMCNKEQVLSVSRAFQINTFNLKVQPFNVTKGQYSTAEECAADSDLNFLIPVAVGVALGFLIIAVFISYMIGRRKSRTGYQSV

SEQ ID NO: 10 - protein, 410 aa, Homo sapiens
MVCFRLFPVPGSGLVLVCLVLGAVRSYALELNLTDSENATCLYAKWQMNFTVRYETTNKTYKTVTISDHGTVTYNGSICGDDQNGPKIAVQFGPGFSWIANFTKAASTYSIDSVSFSYNTGDNTTFPDAEDKGILTVDELLAIRIPLNDLFRCNSLSTLEKNDVVQHYWDVLVQAFVQNGTVSTNEFLCDKDKTSTVAPTIHTTVPSPTTTPTPKEKPEAGTYSVNNGNDTCLLATMGLQLNITQDKVASVININPNTTHSTGSCRSHTALLRLNSSTIKYLDFVFAVKNENRFYLKEVNISMYLVNGSVFSIANNNLSYWDAPLGSSYMCNKEQTVSVSGAFQINTFDLRVQPFNVTQGKYSTAQDCSADDDNFLVPIAVGAALAGVLILVLLAYFIGLKHHHAGYEQF

SEQ ID NO: 11 - protein, 410 aa, Homo sapiens
MVCFRLFPVPGSGLVLVCLVLGAVRSYALELNLTDSENATCLYAKWQMNFTVRYETTNKTYKTVTISDHGTVTYNGSICGDDQNGPKIAVQFGPGFSWIANFTKAASTYSIDSVSFSYNTGDNTTFPDAEDKGILTVDELLAIRIPLNDLFRCNSLSTLEKNDVVQHYWDVLVQAFVQNGTVSTNEFLCDKDKTSTVAPTIHTTVPSPTTTPTPKEKPEAGTYSVNNGNDTCLLATMGLQLNITQDKVASVININPNTTHSTGSCRSHTALLRLNSSTIKYLDFVFAVKNENRFYLKEVNISMYLVNGSVFSIANNNLSYWDAPLGSSYMCNKEQTVSVSGAFQINTFDLRVQPFNVTQGKYSTAQECSLDDDTILIPIIVGAGLSGLIIVIVIAYVIGRRKSYAGYQTL

SEQ ID NO: 12 - protein, 411 aa, Homo sapiens
MVCFRLFPVPGSGLVLVCLVLGAVRSYALELNLTDSENATCLYAKWQMNFTVRYETTNKTYKTVTISDHGTVTYNGSICGDDQNGPKIAVQFGPGFSWIANFTKAASTYSIDSVSFSYNTGDNTTFPDAEDKGILTVDELLAIRIPLNDLFRCNSLSTLEKNDVVQHYWDVLVQAFVQNGTVSTNEFLCDKDKTSTVAPTIHTTVPSPTTTPTPKEKPEAGTYSVNNGNDTCLLATMGLQLNITQDKVASVININPNTTHSTGSCRSHTALLRLNSSTIKYLDFVFAVKNENRFYLKEVNISMYLVNGSVFSIANNNLSYWDAPLGSSYMCNKEQTVSVSGAFQINTFDLRVQPFNVTQGKYSTAEECSADSDLNFLIPVAVGVALGFLIIVVFISYMIGRRKSRTGYQSV